European Patent Application EP 4 582 108 A1, published July 9, 2025. Title: ＨＩＶ感染を治療するための組成物. Applicant: 国立研究開発法人医薬基盤・健康・栄養研究所. Application JP. The sequence listing filed with the application follows.

SEQUENCE LISTING (16 sequences)

SEQ ID NO: 1 - DNA, 978 bp, synthetic construct
  source 1..978: mol_type = other DNA
  CDS <1..978: protein_id = 2; translation = MTDVSGKIRAWGRRLLVGAAAAAALPGLVGLAGGAATAGAFSRPGLPVEYLQVPSAAMGRSIKVQFQSGGDNSPAVYLLDGLRAQDDYNGWDINTPAFEWYYQSGLSVIMPVGGQSSFYSDWYSPACGKAGCTTYKWETFLTSELPQWLSANRSVKPTGSAAVGISMAGSSALILSVYHPQQFIYAGSLSALMDPSQGMGPSLIGLAMGDAGGYKASDMWGPSSDPAWQRNDPSLHIPELVANNTRLWIYCGNGTPSELGGANVPAEFLENFVRSSNLKFQDAYNAAGGHNAVFNLDANGTHSWEYWGAQLNAMKGDLQASLGAR
atgacagacgtgagcgggaagattcgggcgtggggccgacgccttctggtcggcgcggccgctgctgcggcccttcctggcctggtcggactcgccggcggagcggcgaccgcgggagcgttctcccgtcccggcctgccggtggagtacctccaggtgccgtcggctgcgatgggtcgcagtatcaaggttcaattccaaagtggcggggacaactcgccggcggtgtacctgctcgacggtctccgcgctcaagacgactacaacggctgggacatcaacaccccggccttcgagtggtactaccaatcgggcctgtcggtcatcatgccggtcggcggacagtccagtttctacagtgactggtacagcccggcctgcggcaaggccggctgcacgacctacaagtgggagaccttcctgaccagcgagctgccgcaatggctgtccgcgaaccggagtgtcaagcccaccggaagcgccgcggtcggcatctcgatggccggctcgtcggccctgatcctgtccgtctaccacccgcagcagttcatctacgcgggttcgttgtcggccctgatggacccctcccaggggatggggccgtctctgatcggcttggcgatgggtgacgccggtggttacaaggcctcggacatgtggggaccctcgagtgacccagcctggcagcgtaacgacccgtcgctgcacattccggagctggtcgccaacaacacccgcctgtggatctactgcggcaacggcaccccgtccgagttgggcggtgccaatgttccggccgaattcctggagaacttcgttcgcagcagcaacctgaaattccaggacgcctacaacgccgcgggcggccacaacgccgtgttcaatttggacgccaacggaacgcacagctgggagtactggggcgcgcagctcaacgccatgaagggtgacctgcaggccagcctgggcgcccgctga

SEQ ID NO: 2 - protein, 325 aa, synthetic construct
MTDVSGKIRAWGRRLLVGAAAAAALPGLVGLAGGAATAGAFSRPGLPVEYLQVPSAAMGRSIKVQFQSGGDNSPAVYLLDGLRAQDDYNGWDINTPAFEWYYQSGLSVIMPVGGQSSFYSDWYSPACGKAGCTTYKWETFLTSELPQWLSANRSVKPTGSAAVGISMAGSSALILSVYHPQQFIYAGSLSALMDPSQGMGPSLIGLAMGDAGGYKASDMWGPSSDPAWQRNDPSLHIPELVANNTRLWIYCGNGTPSELGGANVPAEFLENFVRSSNLKFQDAYNAAGGHNAVFNLDANGTHSWEYWGAQLNAMKGDLQASLGAR

SEQ ID NO: 3 - DNA, 11022 bp, synthetic construct
  source 1..11022: mol_type = other DNA
gcatgcacattttaaaggcttttgctaaatatagccaaaagtccttctacaaattttctaagagttctgattcaaagcagtaacaggccttgtctcatcatgaactttggcatttcatctacagctaagtttatatcataaatagttctttacaggcagcaccaacttatacccttatagcatactttactgtgtgaaaattgcatctttcattaagcttactgtaaatttactggctgtcttccttgcaggtttctggaagggatttattacagtgcaagaagacatagaatcttagacatatacttagaaaaggaagaaggcatcataccagattggcaggattacacctcaggaccaggaattagatacccaaagacatttggctggctatggaaattagtccctgtaaatgtatcagatgaggcacaggaggatgaggagcattatttaatgcatccagctcaaacttcccagtgggatgacccttggggagaggttctagcatggaagtttgatccaactctggcctacacttatgaggcatatgttagatacccagaagagtttggaagcaagtcaggcctgtcagaggaagaggttagaagaaggctaaccgcaagaggccttcttaacatggctgacaagaaggaaactcgctgaaacagcagggactttccacaaggggatgttacggggaggtactggggaggagccggtcgggaacgcccactttcttgatgtataaatatcactgcatttcgctctgtattcagtcgctctgcggagaggctggcagattgagccctgggaggttctctccagcactagcaggtagagcctgggtgttccctgctagactctcaccagcacttggccggtgctgggcagagtgactccacgcttgcttgcttaaagccctcttcaataaagctgccattttagaagtaagctagtgtgtgttcccatctctcctagccgccgcctggtcaactcggtactcaataataagaagaccctggtctgttaggaccctttctgctttgggaaaccgaagcaggaaaatccctagcagattggcgcctgaacagggacttgaaggagagtgagagactcctgagtacggctgagtgaaggcagtaagggcggcaggaaccaaccacgacggagtgctcctataaaggcgcgggtcggtaccagacggcgtgaggagcgggagaggaagaggcctccggttgcaggtaagtgcaacacaaaaaagaaatagctgtcttttatccaggaaggggtaataagatagagtgggagatgggcgtgagaaactccgtcttgtcagggaagaaagcagatgaattagaaaaaattaggctacgacccaacggaaagaaaaagtacatgttgaagcatgtagtatgggcagcaaatgaattagatagatttggattagcagaaagcctgttggagaacaaagaaggatgtcaaaaaatactttcggtcttagctccattagtgccaacaggctcagaaaatttaaaaagcctttataatactgtctgcgtcatctggtgcattcacgcagaagagaaagtgaaacacactgaggaagcaaaacagatagtgcagagacacctagtggtggaaacaggaacaacagaaactatgccaaaaacaagtagaccaacagcaccatctagcggcagaggaggaaattacccagtacaacaaataggtggtaactatgtccacctgccattaagcccgagaacattaaatgcctgggtaaaattgatagaggaaaagaaatttggagcagaagtagtgccaggatttcaggcactgtcagaaggttgcaccccctatgacattaatcagatgttaaattgtgtgggagaccatcaagcggctatgcagattatcagagatattataaacgaggaggctgcagattgggacttgcagcacccacaaccagctccacaacaaggacaacttagggagccgtcaggatcagatattgcaggaacaactagttcagtagatgaacaaatccagtggatgtacagacaacagaaccccataccagtaggcaacatttacaggagatggatccaactggggttgcaaaaatgtgtcagaatgtataacccaacaaacattctagatgtaaaacaagggccaaaagagccatttcagagctatgtagacaggttctacaaaagtttaagagcagaacagacagatgcagcagtaaagaattggatgactcaaacactgctgattcaaaatgctaacccagattgcaagctagtgctgaaggggctgggtgtgaatcccaccctagaagaaatgctgacggcttgtcaaggagtaggggggccgggacagaaggctagattaatggcagaagccctgaaagaggccctcgcaccagtgccaatcccttttgcagcagcccaacagaggggaccaagaaagccaattaagtgttggaattgtgggaaagagggacactctgcaaggcaatgcagagccccaagaagacagggatgctggaaatgtggaaaaatggaccatgttatggccaaatgcccagacagacaggcgggttttttaggccttggtccatggggaaagaagccccgcaatttccccatggctcaagtgcatcaggggctgatgccaactgctcccccagaggacccagctgtggatctgctaaagaactacatgcagttgggcaagcagcagagagaaaagcagagagaaagcagagagaagccttacaaggaggtgacagaggatttgctgcacctcaattctctctttggaggagaccagtagtcactgctcatattgaaggacagcctgtagaagtattactggatacaggggctgatgattctattgtaacaggaatagagttaggtccacattataccccaaaaatagtaggaggaataggaggttttattaatactaaagaatacaaaaatgtagaaatagaagttttaggcaaaaggattaaagggacaatcatgacaggggacaccccgattaacatttttggtagaaatttgctaacagctctggggatgtctctaaattttcccatagctaaagtagagcctgtaaaagtcgccttaaagccaggaaaggatggaccaaaattgaagcagtggccattatcaaaagaaaagatagttgcattaagagaaatctgtgaaaagatggaaaaggatggtcagttggaggaagctcccccgaccaatccatacaacacccccacatttgctataaagaaaaaggataagaacaaatggagaatgctgatagattttagggaactaaatagggtcactcaggactttacggaagtccaattaggaataccacaccctgcaggactagcaaaaaggaaaagaattacagtactggatataggtgatgcatatttctccatacctctagatgaagaatttaggcagtacactgcctttactttaccatcagtaaataatgcagagccaggaaaacgatacatttataaggttctgcctcagggatggaaggggtcaccagccatcttccaatacactatgagacatgtgctagaacccttcaggaaggcaaatccagatgtgaccttagtccagtatatggatgacatcttaatagctagtgacaggacagacctggaacatgacagggtagttttacagtcaaaggaactcttgaatagcatagggttttctaccccagaagagaaattccaaaaagatcccccatttcaatggatggggtacgaattgtggccaacaaaatggaagttgcaaaagatagagttgccacaaagagagacctggacagtgaatgatatacagaagttagtaggagtattaaattgggcagctcaaatttatccaggtataaaaaccaaacatctctgtaggttaattagaggaaaaatgactctaacagaggaagttcagtggactgagatggcagaagcagaatatgaggaaaataaaataattctcagtcaggaacaagaaggatgttattaccaagaaggcaagccattagaagccacggtaataaagagtcaggacaatcagtggtcttataaaattcaccaagaagacaaaatactgaaagtaggaaaatttgcaaagataaagaatacacataccaatggagtgagactattagcacatgtaatacagaaaataggaaaggaagcaatagtgatctggggacaggtcccaaaattccacttaccagttgagaaggatgtatgggaacagtggtggacagactattggcaggtaacctggataccggaatgggattttatctcaacaccaccgctagtaagattagtcttcaatctagtgaaggaccctatagagggagaagaaacctattatacagatggatcatgtaataaacagtcaaaagaagggaaagcaggatatatcacagataggggcaaagacaaagtaaaagtgttagaacagactactaatcaacaagcagaattggaagcatttctcatggcattgacagactcagggccaaaggcaaatattatagtagattcacaatatgttatgggaataataacaggatgccctacagaatcagagagcaggctagttaatcaaataatagaagaaatgattaaaaagtcagaaatttatgtagcatgggtaccagcacacaaaggtataggaggaaaccaagaaatagaccacctagttagtcaagggattagacaagttctcttcttggaaaagatagagccagcacaagaagaacatgataaataccatagtaatgtaaaagaattggtattcaaatttggattacccagaatagtggccagacagatagtagacacctgtgataaatgtcatcagaaaggagaggctatacatgggcaggcaaattcagatctagggacttggcaaatggattgtacccatctagagggaaaaataatcatagttgcagtacatgtagctagtggattcatagaagcagaggtaattccacaagagacaggaagacagacagcactatttctgttaaaattggcaggcagatggcctattacacatctacacacagataatggtgctaactttgcttcgcaagaagtaaagatggttgcatggtgggcagggatagagcacacctttggggtaccatacaatccacagagtcagggagtagtggaagcaatgaatcaccacctgaaaaatcaaatagatagaatcagggaacaagcaaattcagtagaaaccatagtattaatggcagttcattgcatgaattttaaaagaaggggaggaataggggatatgactccagcagaaagattaattaacatgatcactacagaacaagagatacaatttcaacaatcaaaaaactcaaaatttaaaaattttcgggtctattacagagaaggcagagatcaactgtggaagggacccggtgagctattgtggaaaggggaaggagcagtcatcttaaaggtagggacagacattaaggtagtacccagaagaaaggctaaaattatcaaagattatggaggaggaaaagaggtggatagcagttcccacatggaggataccggagaggctagagaggtggcatagcctcataaaatatctgaaatataaaactaaagatctacaaaaggtttgctatgtgccccattttaaggtcggatgggcatggtggacctgcagcagagtaatcttcccactacaggaaggaagccatttagaagtacaagggtattggcatttgacaccagaaaaagggtggctcagtacttatgcagtgaggataacctggtactcaaagaacttttggacagatgtaacaccaaactatgcagacattttactgcatagcacttatttcccttgctttacagcgggagaagtgagaagggccatcaggggagaacaactgctgtcttgctgcaggttcccgagagctcataagtaccaggtaccaagcctacagtacttagcactgaaagtagtaagcgatgtcagatcccagggagagaatcccacctggaaacagtggagaagagacaataggagaggccttcgaatggctaaacagaacagtagaggagataaacagagaggcggtaaaccacctaccaagggagctaattttccaggtttggcaaaggtcttgggaatactggcatgatgaacaagggatgtcaccaagctatgtaaaatacagatacttgtgtttaatacaaaaggctttatttatgcattgcaagaaaggctgtagatgtctaggggaaggacatggggcagggggatggagaccaggacctcctcctcctccccctccaggactagcataaatggaacaagccccagaagaccaagggccacagagggagccatacaatgaatggacactagagcttttagaggaacttaagagtgaagctgttagacattttcctaggatatggctccataacttaggacaacatatctatgaaacttacggggatacttgggcaggagtggaagccataataagaattctgcaacaactgctgtttatccatttcagaattgggtgtcgacatagcagaataggcgttactcgacagaggagagcaagaaatggagccagtagatcctagactagagccctggaagcatccaggaagtcagcctaaaactgcttgtaccaattgctattgtaaaaagtgttgctttcattgccaagtttgtttcatgacaaaagccttaggcatctcctatggcaggaagaagcggagacagcgacgaagagctcatcagaacagtcagactcatcaagcttctctatcaaagcagtaagtagtacatgtaatgcaacctataatagtagcaatagtagcattagtagtagcaataataatagcaatagttgtgtggtccatagtaatcatagaatataggaaaatattaagacaaagaaaaatagacaggttaattgatagactaatagaaagagcagaagacagtggcaatgagagtgaaggagaagtatcagcacttgtggagatgggggtggaaatggggcaccatgctccttgggatattgatgatctgtagtgctacagaaaaattgtgggtcacagtctattatggggtacctgtgtggaaggaagcaaccaccactctattttgtgcatcagatgctaaagcatatgatacagaggtacataatgtttgggccacacatgcctgtgtacccacagaccccaacccacaagaagtagtattggtaaatgtgacagaaaattttaacatgtggaaaaatgacatggtagaacagatgcatgaggatataatcagtttatgggatcaaagcctaaagccatgtgtaaaattaaccccactctgtgttagtttaaagtgcactgatttgaagaatgatactaataccaatagtagtagcgggagaatgataatggagaaaggagagataaaaaactgctctttcaatatcagcacaagcataagagataaggtgcagaaagaatatgcattcttttataaacttgatatagtaccaatagataataccagctataggttgataagttgtaacacctcagtcattacacaggcctgtccaaaggtatcctttgagccaattcccatacattattgtgccccggctggttttgcgattctaaaatgtaataataagacgttcaatggaacaggaccatgtacaaatgtcagcacagtacaatgtacacatggaatcaggccagtagtatcaactcaactgctgttaaatggcagtctagcagaagaagatgtagtaattagatctgccaatttcacagacaatgctaaaaccataatagtacagctgaacacatctgtagaaattaattgtacaagacccaacaacaatacaagaaaaagtatccgtatccagaggggaccagggagagcatttgttacaataggaaaaataggaaatatgagacaagcacattgtaacattagtagagcaaaatggaatgccactttaaaacagatagctagcaaattaagagaacaatttggaaataataaaacaataatctttaagcaatcctcaggaggggacccagaaattgtaacgcacagttttaattgtggaggggaatttttctactgtaattcaacacaactgtttaatagtacttggtttaatagtacttggagtactgaagggtcaaataacactgaaggaagtgacacaatcacactcccatgcagaataaaacaatttataaacatgtggcaggaagtaggaaaagcaatgtatgcccctcccatcagtggacaaattagatgttcatcaaatattactgggctgctattaacaagagatggtggtaataacaacaatgggtccgagatcttcagacctggaggaggcgatatgagggacaattggagaagtgaattatataaatataaagtagtaaaaattgaaccattaggagtagcacccaccaaggcaaagagaagagtggtgcagagagaaaaaagagcagtgggaataggagctttgttccttgggttcttgggagcagcaggaagcactatgggcgcagcgtcaatgacgctgacggtacaggccagacaattattgtctgatatagtgcagcagcagaacaatttgctgagggctattgaggcgcaacagcatctgttgcaactcacagtctggggcatcaaacagctccaggcaagaatcctggctgtggaaagatacctaaaggatcaacagctcctggggatttggggttgctctggaaaactcatttgcaccactgctgtgccttggaatgctagttggagtaataaatctctggaacagatttggaataacatgacctggatggagtgggacagagaaattaacaattacacaagcttaatacactccttaattgaagaatcgcaaaaccagcaagaaaagaatgaacaagaattattggaattagataaatgggcaagtttgtggaattggtttaacataacaaattggctgtggtatataaaattattcataatgatagtaggaggcttggtaggtttaagaatagtttttgctgtactttctatagtgaatagagttaggcagggatattcaccattatcgtttcagacccacctcccaatcccgaggggacccgacaggcccgaaggaatagaagaagaaggtggagagagagacagagacagatccattcgattagtgaacggatccttagcacttatctgggacgatctgcggagcctgtgcctcttcagctaccaccgcttgagagacttactcttgattgtaacgaggattgtggaacttctgggacgcagggggtgggaagccctcaaatattggtggaatctcctacagtattggagtcaggaactaaagaatagtgctgttaacttgctcaatgccacagccatagcagtagctgaggggacagatagggttatagaagtattacaagcagcttatagagctattcgccacatacctagaagaataagacagggcttggaaaggattttgctataaatgacagacgtgagcgggaagattcgggcgtggggccgacgccttctggtcggcgcggccgctgctgcggcccttcctggcctggtcggactcgccggcggagcggcgaccgcgggagcgttctcccgtcccggcctgccggtggagtacctccaggtgccgtcggctgcgatgggtcgcagtatcaaggttcaattccaaagtggcggggacaactcgccggcggtgtacctgctcgacggtctccgcgctcaagacgactacaacggctgggacatcaacaccccggccttcgagtggtactaccaatcgggcctgtcggtcatcatgccggtcggcggacagtccagtttctacagtgactggtacagcccggcctgcggcaaggccggctgcacgacctacaagtgggagaccttcctgaccagcgagctgccgcaatggctgtccgcgaaccggagtgtcaagcccaccggaagcgccgcggtcggcatctcgatggccggctcgtcggccctgatcctgtccgtctaccacccgcagcagttcatctacgcgggttcgttgtcggccctgatggacccctcccaggggatggggccgtctctgatcggcttggcgatgggtgacgccggtggttacaaggcctcggacatgtggggaccctcgagtgacccagcctggcagcgtaacgacccgtcgctgcacattccggagctggtcgccaacaacacccgcctgtggatctactgcggcaacggcaccccgtccgagttgggcggtgccaatgttccggccgaattcctggagaacttcgttcgcagcagcaacctgaaattccaggacgcctacaacgccgcgggcggccacaacgccgtgttcaatttggacgccaacggaacgcacagctgggagtactggggcgcgcagctcaacgccatgaagggtgacctgcaggccagcctgggcgcccgctgaaacagcagggactttccacaaggggatgttacggggaggtactggggaggagccggtcgggaacgcccactttcttgatgtataaatatcactgcatttcgctctgtattcagtcgctctgcggagaggctggcagattgagccctgggaggttctctccagcactagcaggtagagcctgggtgttccctgctagactctcaccagcacttggccggtgctgggcagagtgactccacgcttgcttgcttaaagccctcttcaataaagctgccattttagaagtaagctagtgtgtgttcccatctctcctagccgccgcctggtcaactcggtactcaataataagaagaccctggtctgttaggaccctttctgctttgggaaaccgaagcaggaaaatccctagca

SEQ ID NO: 4 - DNA, 15182 bp, synthetic construct
  source 1..15182: mol_type = other DNA
tggaagggctaatttggtcccaaaaaagacaagagatccttgatctgtggatctaccacacacaaggctacttccctgattggcagaactacacaccagggccagggatcagatatccactgacctttggatggtgcttcaagttagtaccagttgaaccagagcaagtagaagaggccaatgaaggagagaacaacagcttgttacaccctatgagccagcatgggatggaggacccggagggagaagtattagtgtggaagtttgacagcctcctagcatttcgtcacatggcccgagagctgcatccggagtactacaaagactgctgacatcgagctttctacaagggactttccgctggggactttccagggaggtgtggcctgggcgggactggggagtggcgagccctcagatgctacatataagcagctgctttttgcctgtactgggtctctctggttagaccagatctgagcctgggagctctctggctaactagggaacccactgcttaagcctcaataaagcttgccttgagtgctcaaagtagtgtgtgcccgtctgttgtgtgactctggtaactagagatccctcagacccttttagtcagtgtggaaaatctctagcagtggcgcccgaacagggacttgaaagcgaaagtaaagccagaggagatctctcgacgcaggactcggcttgctgaagcgcgcacggcaagaggcgaggggcggcgactggtgagtacgccaaaaattttgactagcggaggctagaaggagagagatgggtgcgagagcgtcggtattaagcgggggagaattagataaatgggaaaaaattcggttaaggccagggggaaagaaacaatataaactaaaacatatagtatgggcaagcagggagctagaacgattcgcagttaatcctggccttttagagacatcagaaggctgtagacaaatactgggacagctacaaccatcccttcagacaggatcagaagaacttagatcattatataatacaatagcagtcctctattgtgtgcatcaaaggatagatgtaaaagacaccaaggaagccttagataagatagaggaagagcaaaacaaaagtaagaaaaaggcacagcaagcagcagctgacacaggaaacaacagccaggtcagccaaaattaccctatagtgcagaacctccaggggcaaatggtacatcaggccatatcacctagaactttaaatgcatgggtaaaagtagtagaagagaaggctttcagcccagaagtaatacccatgttttcagcattatcagaaggagccaccccacaagatttaaataccatgctaaacacagtggggggacatcaagcagccatgcaaatgttaaaagagaccatcaatgaggaagctgcagaatgggatagattgcatccagtgcatgcagggcctattgcaccaggccagatgagagaaccaaggggaagtgacatagcaggaactactagtacccttcaggaacaaataggatggatgacacataatccacctatcccagtaggagaaatctataaaagatggataatcctgggattaaataaaatagtaagaatgtatagccctaccagcattctggacataagacaaggaccaaaggaaccctttagagactatgtagaccgattctataaaactctaagagccgagcaagcttcacaagaggtaaaaaattggatgacagaaaccttgttggtccaaaatgcgaacccagattgtaagactattttaaaagcattgggaccaggagcgacactagaagaaatgatgacagcatgtcagggagtggggggacccggccataaagcaagagttttggctgaagcaatgagccaagtaacaaatccagctaccataatgatacagaaaggcaattttaggaaccaaagaaagactgttaagtgtttcaattgtggcaaagaagggcacatagccaaaaattgcagggcccctaggaaaaagggctgttggaaatgtggaaaggaaggacaccaaatgaaagattgtactgagagacaggctaattttttagggaagatctggccttcccacaagggaaggccagggaattttcttcagagcagaccagagccaacagccccaccagaagagagcttcaggtttggggaagagacaacaactccctctcagaagcaggagccgatagacaaggaactgtatcctttagcttccctcagatcactctttggcagcgacccctcgtcacaataaagataggggggcaattaaaggaagctctattagatacaggagcagatgatacagtattagaagaaatgaatttgccaggaagatggaaaccaaaaatgatagggggaattggaggttttatcaaagtaagacagtatgatcagatactcatagaaatctgcggacataaagctataggtacagtattagtaggacctacacctgtcaacataattggaagaaatctgttgactcagattggctgcactttaaattttcccattagtcctattgagactgtaccagtaaaattaaagccaggaatggatggcccaaaagttaaacaatggccattgacagaagaaaaaataaaagcattagtagaaatttgtacagaaatggaaaaggaaggaaaaatttcaaaaattgggcctgaaaatccatacaatactccagtatttgccataaagaaaaaagacagtactaaatggagaaaattagtagatttcagagaacttaataagagaactcaagatttctgggaagttcaattaggaataccacatcctgcagggttaaaacagaaaaaatcagtaacagtactggatgtgggcgatgcatatttttcagttcccttagataaagacttcaggaagtatactgcatttaccatacctagtataaacaatgagacaccagggattagatatcagtacaatgtgcttccacagggatggaaaggatcaccagcaatattccagtgtagcatgacaaaaatcttagagccttttagaaaacaaaatccagacatagtcatctatcaatacatggatgatttgtatgtaggatctgacttagaaatagggcagcatagaacaaaaatagaggaactgagacaacatctgttgaggtggggatttaccacaccagacaaaaaacatcagaaagaacctccattcctttggatgggttatgaactccatcctgataaatggacagtacagcctatagtgctgccagaaaaggacagctggactgtcaatgacatacagaaattagtgggaaaattgaattgggcaagtcagatttatgcagggattaaagtaaggcaattatgtaaacttcttaggggaaccaaagcactaacagaagtagtaccactaacagaagaagcagagctagaactggcagaaaacagggagattctaaaagaaccggtacatggagtgtattatgacccatcaaaagacttaatagcagaaatacagaagcaggggcaaggccaatggacatatcaaatttatcaagagccatttaaaaatctgaaaacaggaaagtatgcaagaatgaagggtgcccacactaatgatgtgaaacaattaacagaggcagtacaaaaaatagccacagaaagcatagtaatatggggaaagactcctaaatttaaattacccatacaaaaggaaacatgggaagcatggtggacagagtattggcaagccacctggattcctgagtgggagtttgtcaatacccctcccttagtgaagttatggtaccagttagagaaagaacccataataggagcagaaactttctatgtagatggggcagccaatagggaaactaaattaggaaaagcaggatatgtaactgacagaggaagacaaaaagttgtccccctaacggacacaacaaatcagaagactgagttacaagcaattcatctagctttgcaggattcgggattagaagtaaacatagtgacagactcacaatatgcattgggaatcattcaagcacaaccagataagagtgaatcagagttagtcagtcaaataatagagcagttaataaaaaaggaaaaagtctacctggcatgggtaccagcacacaaaggaattggaggaaatgaacaagtagataaattggtcagtgctggaatcaggaaagtactatttttagatggaatagataaggcccaagaagaacatgagaaatatcacagtaattggagagcaatggctagtgattttaacctaccacctgtagtagcaaaagaaatagtagccagctgtgataaatgtcagctaaaaggggaagccatgcatggacaagtagactgtagcccaggaatatggcagctagattgtacacatttagaaggaaaagttatcttggtagcagttcatgtagccagtggatatatagaagcagaagtaattccagcagagacagggcaagaaacagcatacttcctcttaaaattagcaggaagatggccagtaaaaacagtacatacagacaatggcagcaatttcaccagtactacagttaaggccgcctgttggtgggcggggatcaagcaggaatttggcattccctacaatccccaaagtcaaggagtaatagaatctatgaataaagaattaaagaaaattataggacaggtaagagatcaggctgaacatcttaagacagcagtacaaatggcagtattcatccacaattttaaaagaaaaggggggattggggggtacagtgcaggggaaagaatagtagacataatagcaacagacatacaaactaaagaattacaaaaacaaattacaaaaattcaaaattttcgggtttattacagggacagcagagatccagtttggaaaggaccagcaaagctcctctggaaaggtgaaggggcagtagtaatacaagataatagtgacataaaagtagtgccaagaagaaaagcaaagatcatcagggattatggaaaacagatggcaggtgatgattgtgtggcaagtagacaggatgaggattaacacatggaaaagattagtaaaacaccatatgtatatttcaaggaaagctaaggactggttttatagacatcactatgaaagtactaatccaaaaataagttcagaagtacacatcccactaggggatgctaaattagtaataacaacatattggggtctgcatacaggagaaagagactggcatttgggtcagggagtctccatagaatggaggaaaaagagatatagcacacaagtagaccctgacctagcagaccaactaattcatctgcactattttgattgtttttcagaatctgctataagaaataccatattaggacgtatagttagtcctaggtgtgaatatcaagcaggacataacaaggtaggatctctacagtacttggcactagcagcattaataaaaccaaaacagataaagccacctttgcctagtgttaggaaactgacagaggacagatggaacaagccccagaagaccaagggccacagagggagccatacaatgaatggacactagagcttttagaggaacttaagagtgaagctgttagacattttcctaggatatggctccataacttaggacaacatatctatgaaacttacggggatacttgggcaggagtggaagccataataagaattctgcaacaactgctgtttatccatttcagaattgggtgtcgacatagcagaataggcgttactcgacagaggagagcaagaaatggagccagtagatcctagactagagccctggaagcatccaggaagtcagcctaaaactgcttgtaccaattgctattgtaaaaagtgttgctttcattgccaagtttgtttcatgacaaaagccttaggcatctcctatggcaggaagaagcggagacagcgacgaagagctcatcagaacagtcagactcatcaagcttctctatcaaagcagtaagtagtacatgtaatgcaacctataatagtagcaatagtagcattagtagtagcaataataatagcaatagttgtgtggtccatagtaatcatagaatataggaaaatattaagacaaagaaaaatagacaggttaattgatagactaatagaaagagcagaagacagtggcaatgagagtgaaggagaagtatcagcacttgtggagatgggggtggaaatggggcaccatgctccttgggatattgatgatctgtagtgctacagaaaaattgtgggtcacagtctattatggggtacctgtgtggaaggaagcaaccaccactctattttgtgcatcagatgctaaagcatatgatacagaggtacataatgtttgggccacacatgcctgtgtacccacagaccccaacccacaagaagtagtattggtaaatgtgacagaaaattttaacatgtggaaaaatgacatggtagaacagatgcatgaggatataatcagtttatgggatcaaagcctaaagccatgtgtaaaattaaccccactctgtgttagtttaaagtgcactgatttgaagaatgatactaataccaatagtagtagcgggagaatgataatggagaaaggagagataaaaaactgctctttcaatatcagcacaagcataagagataaggtgcagaaagaatatgcattcttttataaacttgatatagtaccaatagataataccagctataggttgataagttgtaacacctcagtcattacacaggcctgtccaaaggtatcctttgagccaattcccatacattattgtgccccggctggttttgcgattctaaaatgtaataataagacgttcaatggaacaggaccatgtacaaatgtcagcacagtacaatgtacacatggaatcaggccagtagtatcaactcaactgctgttaaatggcagtctagcagaagaagatgtagtaattagatctgccaatttcacagacaatgctaaaaccataatagtacagctgaacacatctgtagaaattaattgtacaagacccaacaacaatacaagaaaaagtatccgtatccagaggggaccagggagagcatttgttacaataggaaaaataggaaatatgagacaagcacattgtaacattagtagagcaaaatggaatgccactttaaaacagatagctagcaaattaagagaacaatttggaaataataaaacaataatctttaagcaatcctcaggaggggacccagaaattgtaacgcacagttttaattgtggaggggaatttttctactgtaattcaacacaactgtttaatagtacttggtttaatagtacttggagtactgaagggtcaaataacactgaaggaagtgacacaatcacactcccatgcagaataaaacaatttataaacatgtggcaggaagtaggaaaagcaatgtatgcccctcccatcagtggacaaattagatgttcatcaaatattactgggctgctattaacaagagatggtggtaataacaacaatgggtccgagatcttcagacctggaggaggcgatatgagggacaattggagaagtgaattatataaatataaagtagtaaaaattgaaccattaggagtagcacccaccaaggcaaagagaagagtggtgcagagagaaaaaagagcagtgggaataggagctttgttccttgggttcttgggagcagcaggaagcactatgggcgcagcgtcaatgacgctgacggtacaggccagacaattattgtctgatatagtgcagcagcagaacaatttgctgagggctattgaggcgcaacagcatctgttgcaactcacagtctggggcatcaaacagctccaggcaagaatcctggctgtggaaagatacctaaaggatcaacagctcctggggatttggggttgctctggaaaactcatttgcaccactgctgtgccttggaatgctagttggagtaataaatctctggaacagatttggaataacatgacctggatggagtgggacagagaaattaacaattacacaagcttaatacactccttaattgaagaatcgcaaaaccagcaagaaaagaatgaacaagaattattggaattagataaatgggcaagtttgtggaattggtttaacataacaaattggctgtggtatataaaattattcataatgatagtaggaggcttggtaggtttaagaatagtttttgctgtactttctatagtgaatagagttaggcagggatattcaccattatcgtttcagacccacctcccaatcccgaggggacccgacaggcccgaaggaatagaagaagaaggtggagagagagacagagacagatccattcgattagtgaacggatccttagcacttatctgggacgatctgcggagcctgtgcctcttcagctaccaccgcttgagagacttactcttgattgtaacgaggattgtggaacttctgggacgcagggggtgggaagccctcaaatattggtggaatctcctacagtattggagtcaggaactaaagaatagtgctgttaacttgctcaatgccacagccatagcagtagctgaggggacagatagggttatagaagtattacaagcagcttatagagctattcgccacatacctagaagaataagacagggcttggaaaggattttgctataagatgacagacgtgagcgggaagattcgggcgtggggccgacgccttctggtcggcgcggccgctgctgcggcccttcctggcctggtcggactcgccggcggagcggcgaccgcgggagcgttctcccgtcccggcctgccggtggagtacctccaggtgccgtcggctgcgatgggtcgcagtatcaaggttcaattccaaagtggcggggacaactcgccggcggtgtacctgctcgacggtctccgcgctcaagacgactacaacggctgggacatcaacaccccggccttcgagtggtactaccaatcgggcctgtcggtcatcatgccggtcggcggacagtccagtttctacagtgactggtacagcccggcctgcggcaaggccggctgcacgacctacaagtgggagaccttcctgaccagcgagctgccgcaatggctgtccgcgaaccggagtgtcaagcccaccggaagcgccgcggtcggcatctcgatggccggctcgtcggccctgatcctgtccgtctaccacccgcagcagttcatctacgcgggttcgttgtcggccctgatggacccctcccaggggatggggccgtctctgatcggcttggcgatgggtgacgccggtggttacaaggcctcggacatgtggggaccctcgagtgacccagcctggcagcgtaacgacccgtcgctgcacattccggagctggtcgccaacaacacccgcctgtggatctactgcggcaacggcaccccgtccgagttgggcggtgccaatgttccggccgaattcctggagaacttcgttcgcagcagcaacctgaaattccaggacgcctacaacgccgcgggcggccacaacgccgtgttcaatttggacgccaacggaacgcacagctgggagtactggggcgcgcagctcaacgccatgaagggtgacctgcaggccagcctgggcgcccgctgacatcgagcttgctacaagggactttccgctggggactttccagggaggcgtggcctgggcgggactggggagtggcgagccctcagatgctgcatataagcagctgctttttgcctgtactgggtctctctggttagaccagatctgagcctgggagctctctggctaactagggaacccactgcttaagcctcaataaagcttgccttgagtgcttcaagtagtgtgtgcccgtctgttgtgtgactctggtaactagagatccctcagacccttttagtcagtgtggaaaatctctagcacccaggaggtagaggttgcagtgagccaagatcgcgccactgcattccagcctgggcaagaaaacaagactgtctaaaataataataataagttaagggtattaaatatatttatacatggaggtcataaaaatatatatatttgggctgggcgcagtggctcacacctgcgcccggccctttgggaggccgaggcaggtggatcacctgagtttgggagttccagaccagcctgaccaacatggagaaaccccttctctgtgtatttttagtagattttattttatgtgtattttattcacaggtatttctggaaaactgaaactgtttttcctctactctgataccacaagaatcatcagcacagaggaagacttctgtgatcaaatgtggtgggagagggaggttttcaccagcacatgagcagtcagttctgccgcagactcggcgggtgtccttcggttcagttccaacaccgcctgcctggagagaggtcagaccacagggtgagggctcagtccccaagacataaacacccaagacataaacacccaacaggtccaccccgcctgctgcccaggcagagccgattcaccaagacgggaattaggatagagaaagagtaagtcacacagagccggctgtgcgggagaacggagttctattatgactcaaatcagtctccccaagcattcggggatcagagtttttaaggataacttagtgtgtagggggccagtgagttggagatgaaagcgtagggagtcgaaggtgtccttttgcgccgagtcagttcctgggtgggggccacaagatcggatgagccagtttatcaatccgggggtgccagctgatccatggagtgcagggtctgcaaaatatctcaagcactgattgatcttaggttttacaatagtgatgttaccccaggaacaatttggggaaggtcagaatcttgtagcctgtagctgcatgactcctaaaccataatttcttttttgtttttttttttttatttttgagacagggtctcactctgtcacctaggctggagtgcagtggtgcaatcacagctcactgcagcctcaacgtcgtaagctcaagcgatcctcccacctcagcctgcctggtagctgagactacaagcgacgccccagttaatttttgtatttttggtagaggcagcgttttgccgtgtggccctggctggtctcgaactcctgggctcaagtgatccagcctcagcctcccaaagtgctgggacaaccggggccagtcactgcacctggccctaaaccataatttctaatcttttggctaatttgttagtcctacaaaggcagtctagtccccaggcaaaaagggggtttgtttcgggaaagggctgttactgtctttgtttcaaactataaactaagttcctcctaaacttagttcggcctacacccaggaatgaacaaggagagcttggaggttagaagcacgatggaattggttaggtcagatctctttcactgtctgagttataattttgcaatggtggttcaaagactgcccgcttctgacaccagtcgctgcattaatgaatcggccaacgcgcggggagaggcggtttgcgtattgggcgctcttccgcttcctcgctcactgactcgctgcgctcggtcgttcggctgcggcgagcggtatcagctcactcaaaggcggtaatacggttatccacagaatcaggggataacgcaggaaagaacatgtgagcaaaaggccagcaaaaggccaggaaccgtaaaaaggccgcgttgctggcgtttttccataggctccgcccccctgacgagcatcacaaaaatcgacgctcaagtcagaggtggcgaaacccgacaggactataaagataccaggcgtttccccctggaagctccctcgtgcgctctcctgttccgaccctgccgcttaccggatacctgtccgcctttctcccttcgggaagcgtggcgctttctcatagctcacgctgtaggtatctcagttcggtgtaggtcgttcgctccaagctgggctgtgtgcacgaaccccccgttcagcccgaccgctgcgccttatccggtaactatcgtcttgagtccaacccggtaagacacgacttatcgccactggcagcagccactggtaacaggattagcagagcgaggtatgtaggcggtgctacagagttcttgaagtggtggcctaactacggctacactagaagaacagtatttggtatctgcgctctgctgaagccagttaccttcggaaaaagagttggtagctcttgatccggcaaacaaaccaccgctggtagcggtggtttttttgtttgcaagcagcagattacgcgcagaaaaaaaggatctcaagaagatcctttgatcttttctacggggtctgacgctcagtggaacgaaaactcacgttaagggattttggtcatgagattatcaaaaaggatcttcacctagatccttttaaattaaaaatgaagttttaaatcaatctaaagtatatatgagtaaacttggtctgacagttaccaatgcttaatcagtgaggcacctatctcagcgatctgtctatttcgttcatccatagttgcctgactccccgtcgtgtagataactacgatacgggagggcttaccatctggccccagtgctgcaatgataccgcgagacccacgctcaccggctccagatttatcagcaataaaccagccagccggaagggccgagcgcagaagtggtcctgcaactttatccgcctccatccagtctattaattgttgccgggaagctagagtaagtagttcgccagttaatagtttgcgcaacgttgttgccattgctacaggcatcgtggtgtcacgctcgtcgtttggtatggcttcattcagctccggttcccaacgatcaaggcgagttacatgatcccccatgttgtgcaaaaaagcggttagctccttcggtcctccgatcgttgtcagaagtaagttggccgcagtgttatcactcatggttatggcagcactgcataattctcttactgtcatgccatccgtaagatgcttttctgtgactggtgagtactcaaccaagtcattctgagaatagtgtatgcggcgaccgagttgctcttgcccggcgtcaatacgggataataccgcgccacatagcagaactttaaaagtgctcatcattggaaaacgttcttcggggcgaaaactctcaaggatcttaccgctgttgagatccagttcgatgtaacccactcgtgcacccaactgatcttcagcatcttttactttcaccagcgtttctgggtgagcaaaaacaggaaggcaaaatgccgcaaaaaagggaataagggcgacacggaaatgttgaatactcatactcttcctttttcaatattattgaagcatttatcagggttattgtctcatgagcggatacatatttgaatgtatttagaaaaataaacaaataggggttccgcgcacatttccccgaaaagtgccacctgacgtctaagaaaccattattatcatgacattaacctataaaaataggcgtatcacgaggccctttcgtctcgcgcgtttcggtgatgacggtgaaaacctctgacacatgcagctcccggagacggtcacagcttgtctgtaagcggatgccgggagcagacaagcccgtcagggcgcgtcagcgggtgttggcgggtgtcggggctggcttaactatgcggcatcagagcagattgtactgagagtgcaccatatgcggtgtgaaataccgcacagatgcgtaaggagaaaataccgcatcaggcgccattcgccattcaggctgcgcaactgttgggaagggcgatcggtgcgggcctcttcgctattacgccaggggaggcagagattgcagtaagctgagatcgcagcactgcactccagcctgggcgacagagtaagactctgtctcaaaaataaaataaataaatcaatcagatattccaatcttttcctttatttatttatttattttctattttggaaacacagtccttccttattccagaattacacatatattctatttttctttatatgctccagttttttttagaccttcacctgaaatgtgtgtatacaaaatctaggccagtccagcagagcctaaaggtaaaaaataaaataataaaaaataaataaaatctagctcactccttcacatcaaaatggagatacagctgttagcattaaataccaaataacccatcttgtcctcaataattttaagcgcctctctccaccacatctaactcctgtcaaaggcatgtgccccttccgggcgctctgctgtgctgccaaccaactggcatgtggactctgcagggtccctaactgccaagccccacagtgtgccctgaggctgccccttccttctagcggctgcccccactcggctttgctttccctagtttcagttacttgcgttcagccaaggtctgaaactaggtgcgcacagagcggtaagactgcgagagaaagagaccagctttacagggggtttatcacagtgcaccctgacagtcgtcagcctcacagggggtttatcacattgcaccctgacagtcgtcagcctcacagggggtttatcacagtgcacccttacaatcattccatttgattcacaatttttttagtctctactgtgcctaacttgtaagttaaatttgatcagaggtgtgttcccagaggggaaaacagtatatacagggttcagtactatcgcatttcaggcctccacctgggtcttggaatgtgtcccccgaggggtgatgactacctcagttggatctccacaggtcacagtgacacaagataaccaagacacctcccaaggctaccacaatgggccgccctccacgtgcacatggccggaggaactgccatgtcggaggtgcaagcacacctgcgcatcagagtccttggtgtggagggagggaccagcgcagcttccagccatccacctgatgaacagaacctagggaaagccccagttctacttacaccaggaaaggc

SEQ ID NO: 5 - DNA, 31 bp, synthetic construct
  source 1..31: mol_type = other DNA
atatcgataccatgttctcccgtcccgggct

SEQ ID NO: 6 - DNA, 27 bp, synthetic construct
  source 1..27: mol_type = other DNA
agggcccctagcgggcgcccaggctgg

SEQ ID NO: 7 - DNA, 22 bp, synthetic construct
  source 1..22: mol_type = other DNA
ccattagtgccaacaggctcag

SEQ ID NO: 8 - DNA, 22 bp, synthetic construct
  source 1..22: mol_type = other DNA
ccccagttggatccatctcctg

SEQ ID NO: 9 - DNA, 20 bp, synthetic construct
  source 1..20: mol_type = other DNA
actgtctgcgtcatctggtg

SEQ ID NO: 10 - DNA, 21 bp, synthetic construct
  source 1..21: mol_type = other DNA
gtcccaatctgcagcctcctc

SEQ ID NO: 11 - DNA, 24 bp, synthetic construct
  source 1..24: mol_type = other DNA
tgtccacctgccattaagtcccga

SEQ ID NO: 12 - DNA, 24 bp, synthetic construct
  source 1..24: mol_type = other DNA
tggaagaaagacctccagaaaatg

SEQ ID NO: 13 - DNA, 24 bp, synthetic construct
  source 1..24: mol_type = other DNA
caagtgcagttagcaagcgaggat

SEQ ID NO: 14 - DNA, 20 bp, synthetic construct
  source 1..20: mol_type = other DNA
tgtgctccggcagttctaca

SEQ ID NO: 15 - DNA, 20 bp, synthetic construct
  source 1..20: mol_type = other DNA
ccgtttcaggaatcggatca

SEQ ID NO: 16 - DNA, 25 bp, synthetic construct
  source 1..25: mol_type = other DNA
tgcacagcagttccacaggcacaag